European Patent Application EP 4 253 415 A1, published October 4, 2023. Title: ANTIBODY AND PREPARATION METHOD THEREFOR. Applicant: MABWELL (SHANGHAI) BIOSCIENCE CO., LTD. The sequence listing filed with the application follows.

SEQUENCE LISTING (87 sequences)

SEQ ID NO: 1 - protein, 107 aa, Artificial Sequence
  Light chain variable region of hz182L
DIQMTQSPSSLSASVGDRVTITCRASQDISNYLNWYQQKPGKAPKLLLYYTSRLHSGVPSRFSGSGSGTDYTLTISSLQPEDFATYFCQQGAGRPYTFGGGTKVEIK

SEQ ID NO: 2 - DNA, 321 bp, Artificial Sequence
  Coding nucleotide sequence of hz182L
gacatccagatgacccagtctccctcctctctgtctgcctccgtgggcgacagagtgaccatcacctgcagagcctcccaggacatctccaactacctgaactggtaccagcagaagcctggcaaggctcccaagctgctgctgtactacacctccaggctgcactccggagtgccctctcggttctctggctccggctctggcaccgactacaccctgaccatctcctccctgcagcccgaggacttcgccacctacttctgccagcagggcgctggacggccctacaccttcggaggaggcaccaaggtggagatcaag

SEQ ID NO: 3 - protein, 117 aa, Artificial Sequence
  Heavy chain variable region hz182-H
QLVQSGAEVKKPGATVKISCKVSGFNIKDIYMHWVQQAPGKGLEWMGRIDPANANTKYDPKFQDRVTITADTSTNTAYMELSSLRSEDTAVYYCASGQLGPLGFDYWGQGTTVTVSS

SEQ ID NO: 4 - DNA, 357 bp, Artificial Sequence
  Coding nucleotide sequence of hz182-H
gaggtgcagctggtgcagtccggagccgaggtgaagaagcctggagccaccgtgaagatctcctgcaaggtgtccggcttcaacatcaaggacatctacatgcactgggtgcagcaggctcctggcaagggcctggagtggatgggacggatcgaccctgccaacgccaacaccaagtacgaccccaagttccaggaccgggtgaccatcaccgctgacacctccaccaacaccgcctacatggagctgtcctccctgcggtccgaggacaccgctgtgtactactgcgcctctggccagctgggacctctgggcttcgactactggggacagggcaccaccgtgaccgtgtcctcc

SEQ ID NO: 5 - protein, 107 aa, Artificial Sequence
  Light chain variable region of humanized 140
DIQMTQSPSSLSASVGDRVTITCRASQDITNYLNWYQQKPGKAPKLLIYYTSRLHSGVPSRFSGSGSGTDYTFTISSLQPEDIATYFCQQGDTFPRTFGGGTKVEIK

SEQ ID NO: 6 - DNA, 321 bp, Artificial Sequence
  Coding nucleotide sequence
gacatccagatgacccagtctccctcctccctgtccgcctccgtgggcgacagggtgaccatcacctgcagagcctcccaggacatcaccaactacctgaactggtaccagcagaagcctggcaaggctcccaagctgctgatctactacacctctcggctgcactccggagtgccctctcggttctccggctctggctctggcaccgactacaccttcaccatctcctccctgcagcccgaggacatcgccacctacttctgccagcagggcgacaccttccctcggaccttcggcggaggcaccaaggtggagatcaag

SEQ ID NO: 7 - protein, 107 aa, Artificial Sequence [sequence omitted]

SEQ ID NO: 8 - protein, 124 aa, Artificial Sequence
  Heavy chain variable region of hz140-H
QVQLVQSGAEVKKPGASVKVSCKASGYKFTNYVMHWVRQAPGQRLEWMGYINPYNDGIKYNEKFTGRVTITRDTSASTAYMELSSLRSEDTAVYYCAREGDFYANYGRLGFAYWGQGTLVTVSS

SEQ ID NO: 9 - DNA, 372 bp, Artificial Sequence
  Coding nucleotide sequence
caggtgcagctggtgcagtccggagccgaggtgaagaagcctggagcctccgtgaaggtgtcctgcaaggcctccggctacaagttcaccaactacgtgatgcactgggtgcggcaggctcctggccagaggctggagtggatgggctacatcaacccttacaacgacggcatcaagtacaacgagaagttcaccggacgggtgaccatcaccagggacacctccgcctccaccgcctacatggagctgtcctccctgcggtccgaggacaccgccgtgtactactgcgctcgggagggcgacttctacgccaactacggacggctgggcttcgcctactggggacagggcaccctggtgaccgtgtcctcc

SEQ ID NO: 10 - protein, 327 aa, Artificial Sequence
  Heavy chain constant region
ASTKGPSVFPLAPCSRSTSESTAALGCLVKDYFPEPVTVSWNSGALTSGVHTFPAVLQSSGLYSLSSVVTVPSSSLGTKTYTCNVDHKPSNTKVDKRVESKYGPPCPPCPAPEFLGGPSVFLFPPKPKDTLMISRTPEVTCVVVDVSQEDPEVQFNWYVDGVEVHNAKTKPREEQFNSTYRVVSVLTVLHQDWLNGKEYKCKVSNKGLPSSIEKTISKAKGQPREPQVYTLPPSQEEMTKNQVSLTCLVKGFYPSDIAVEWESNGQPENNYKTTPPVLDSDGSFFLYSRLTVDKSRWQEGNVFSCSVMHEALHNHYTQKSLSLSLGK

SEQ ID NO: 11 - protein, 124 aa, Artificial Sequence
  Heavy chain variable region
QVQLVQSGAEVKKPGASVKVSCKASGYTFTNYVMHWVRQAPGQRLEWMGYINPYNDGIKYNEKFTGRVTITRDTSASTAYMELSSLRSEDTAVYYCAREGDFYANYGRLGFAYWGQGTLVTVSS

SEQ ID NO: 12 - protein, 124 aa, Artificial Sequence
  Heavy chain variable region
QVQLVQSGAEVKKPGASVKVSCKASGYKFTSYVMHWVRQAPGQRLEWMGYINPYNDGIKYNEKFTGRVTITRDTSASTAYMELSSLRSEDTAVYYCAREGDFYANYGRLGFAYWGQGTLVTVSS

SEQ ID NO: 13 - protein, 124 aa, Artificial Sequence
  Heavy chain variable region
QVQLVQSGAEVKKPGASVKVSCKASGYKFTNYAMHWVRQAPGQRLEWMGYINPYNDGIKYNEKFTGRVTITRDTSASTAYMELSSLRSEDTAVYYCAREGDFYANYGRLGFAYWGQGTLVTVSS

SEQ ID NO: 14 - protein, 124 aa, Artificial Sequence
  Heavy chain variable region
QVQLVQSGAEVKKPGASVKVSCKASGYKFTNYVMSWVRQAPGQRLEWMGYINPYNDGIKYNEKFTGRVTITRDTSASTAYMELSSLRSEDTAVYYCAREGDFYANYGRLGFAYWGQGTLVTVSS

SEQ ID NO: 15 - protein, 124 aa, Artificial Sequence
  Heavy chain variable region
QVQLVQSGAEVKKPGASVKVSCKASGYKFTNYVMHWVRQAPGQRLEWMGWINPYNDGIKYNEKFTGRVTITRDTSASTAYMELSSLRSEDTAVYYCAREGDFYANYGRLGFAYWGQGTLVTVSS

SEQ ID NO: 16 - protein, 124 aa, Artificial Sequence
  Heavy chain variable region
QVQLVQSGAEVKKPGASVKVSCKASGYKFTNYVMHWVRQAPGQRLEWMGYINPGNDGIKYNEKFTGRVTITRDTSASTAYMELSSLRSEDTAVYYCAREGDFYANYGRLGFAYWGQGTLVTVSS

SEQ ID NO: 17 - protein, 124 aa, Artificial Sequence
  Heavy chain variable region
QVQLVQSGAEVKKPGASVKVSCKASGYKFTNYVMHWVRQAPGQRLEWMGYINPYNDGIKYNEKFQGRVTITRDTSASTAYMELSSLRSEDTAVYYCAREGDFYANYGRLGFAYWGQGTLVTVSS

SEQ ID NO: 18 - protein, 124 aa, Artificial Sequence
  Heavy chain variable region
QVQLVQSGAEVKKPGASVKVSCKASGYKFTNYVMHWVRQAPGQRLEWMGYINPYNDGIKYNEKFTGRVTITRDTSASTAYMELSSLRSEDTAVYYCAREGDFYANYGRLGFDYWGQGTLVTVSS

SEQ ID NO: 19 - protein, 124 aa, Artificial Sequence
  Heavy chain variable region
QVQLVQSGAEVKKPGASVKVSCKASGYKFTNYVMHWVRQAPGQRLEWMGYINPYNDAIKYNEKFTGRVTITRDTSASTAYMELSSLRSEDTAVYYCAREGDFYANYGRLGFAYWGQGTLVTVSS

SEQ ID NO: 20 - protein, 78 aa, Artificial Sequence
  Heavy chain variable region
WMGYINPYNEGIKYNEKFTGRVTITRDTSASTAYMELSSLRSEDTAVYYCAREGDFYANYGRLGFAYWGQGTLVTVSS

SEQ ID NO: 21 - protein, 124 aa, Artificial Sequence
  Heavy chain variable region
QVQLVQSGAEVKKPGASVKVSCKASGYKFTNYVMSWVRQAPGQRLEWMGYINPYNDAIKYNEKFTGRVTITRDTSASTAYMELSSLRSEDTAVYYCAREGDFYANYGRLGFAYWGQGTLVTVSS

SEQ ID NO: 22 - protein, 124 aa, Artificial Sequence
  Heavy chain variable region
QVQLVQSGAEVKKPGASVKVSCKASGYTFTNYVMSWVRQAPGQRLEWMGYINPYNDAIKYNEKFTGRVTITRDTSASTAYMELSSLRSEDTAVYYCAREGDFYANYGRLGFAYWGQGTLVTVSS

SEQ ID NO: 23 - protein, 124 aa, Artificial Sequence
  Heavy chain variable region
EVQLVQSGAEVKKPGASVKVSCKASGYKFTNYVMSWVRQAPGQRLEWMGYINPYNDAIKYNEKFTGRVTITRDTSASTAYMELSSLRSEDTAVYYCAREGDFYANYGRLGFAYWGQGTLVTVSS

SEQ ID NO: 24 - protein, 214 aa, Artificial Sequence
  Light chain variable region
DIQMTQSPSSLSASVGDRVTITCRASQDISNYLNWYQQKPGKAPKLLIYYTSRLHSGVPSRFSGSGSGTDYTLTISSLQPEDFATYFCQQGAGRPYTFGGGTKVEIKRTVAAPSVFIFPPSDEQLKSGTASVVCLLNNFYPREAKVQWKVDNALQSGNSQESVTEQDSKDSTYSLSSTLTLSKADYEKHKVYACEVTHQGLSSPVTKSFNRGEC

SEQ ID NO: 25 - protein, 214 aa, Artificial Sequence
  Light chain variable region
DIQMTQSPSSLSASVGDRVTITCRASQDISNYLNWYQQKPGKAPKLLLYYTSRLHSGVPSRFSGSGSGTDYTFTISSLQPEDFATYFCQQGAGRPYTFGGGTKVEIKRTVAAPSVFIFPPSDEQLKSGTASVVCLLNNFYPREAKVQWKVDNALQSGNSQESVTEQDSKDSTYSLSSTLTLSKADYEKHKVYACEVTHQGLSSPVTKSFNRGEC

SEQ ID NO: 26 - protein, 214 aa, Artificial Sequence
  Light chain variable region
DIQMTQSPSSLSASVGDRVTITCRASQDISNYLNWYQQKPGKAPKLLLYYTSRLHSGVPSRFSGSGSGTDYTLTISSLQPEDIATYFCQQGAGRPYTFGGGTKVEIKRTVAAPSVFIFPPSDEQLKSGTASVVCLLNNFYPREAKVQWKVDNALQSGNSQESVTEQDSKDSTYSLSSTLTLSKADYEKHKVYACEVTHQGLSSPVTKSFNRGEC

SEQ ID NO: 27 - protein, 214 aa, Artificial Sequence
  Light chain variable region
DIQMTQSPSSLSASVGDRVTITCRASQDITNYLNWYQQKPGKAPKLLLYYTSRLHSGVPSRFSGSGSGTDYTLTISSLQPEDFATYFCQQGAGRPYTFGGGTKVEIKRTVAAPSVFIFPPSDEQLKSGTASVVCLLNNFYPREAKVQWKVDNALQSGNSQESVTEQDSKDSTYSLSSTLTLSKADYEKHKVYACEVTHQGLSSPVTKSFNRGEC

SEQ ID NO: 28 - protein, 214 aa, Artificial Sequence
  Light chain variable region
DIQMTQSPSSLSASVGDRVTITCRASQDISNYLNWYQQKPGKAPKLLLYYTSRLHSGVPSRFSGSGSGTDYTLTISSLQPEDFATYFCQQGDGRPYTFGGGTKVEIKRTVAAPSVFIFPPSDEQLKSGTASVVCLLNNFYPREAKVQWKVDNALQSGNSQESVTEQDSKDSTYSLSSTLTLSKADYEKHKVYACEVTHQGLSSPVTKSFNRGEC

SEQ ID NO: 29 - protein, 214 aa, Artificial Sequence
  Light chain variable region
DIQMTQSPSSLSASVGDRVTITCRASQDISNYLNWYQQKPGKAPKLLLYYTSRLHSGVPSRFSGSGSGTDYTLTISSLQPEDFATYFCQQGATRPYTFGGGTKVEIKRTVAAPSVFIFPPSDEQLKSGTASVVCLLNNFYPREAKVQWKVDNALQSGNSQESVTEQDSKDSTYSLSSTLTLSKADYEKHKVYACEVTHQGLSSPVTKSFNRGEC

SEQ ID NO: 30 - protein, 214 aa, Artificial Sequence
  Light chain variable region
DIQMTQSPSSLSASVGDRVTITCRASQDISNYLNWYQQKPGKAPKLLLYYTSRLHSGVPSRFSGSGSGTDYTLTISSLQPEDFATYFCQQGAGFPYTFGGGTKVEIKRTVAAPSVFIFPPSDEQLKSGTASVVCLLNNFYPREAKVQWKVDNALQSGNSQESVTEQDSKDSTYSLSSTLTLSKADYEKHKVYACEVTHQGLSSPVTKSFNRGEC

SEQ ID NO: 31 - protein, 214 aa, Artificial Sequence
  Light chain variable region
DIQMTQSPSSLSASVGDRVTITCRASQDISNYLNWYQQKPGKAPKLLLYYTSRLHSGVPSRFSGSGSGTDYTLTISSLQPEDFATYFCQQGAGRPRTFGGGTKVEIKRTVAAPSVFIFPPSDEQLKSGTASVVCLLNNFYPREAKVQWKVDNALQSGNSQESVTEQDSKDSTYSLSSTLTLSKADYEKHKVYACEVTHQGLSSPVTKSFNRGEC

SEQ ID NO: 32 - protein, 214 aa, Artificial Sequence
  Light chain variable region
DIQMTQSPSSLSASVGDRVTITCRASQDISNYLNWYQQKPGKAPKLLLYYTSRLHSGVPSRFSGSGSGTDYTLTISSLQPEDFATYFCQQGDTFPYTFGGGTKVEIKRTVAAPSVFIFPPSDEQLKSGTASVVCLLNNFYPREAKVQWKVDNALQSGNSQESVTEQDSKDSTYSLSSTLTLSKADYEKHKVYACEVTHQGLSSPVTKSFNRGEC

SEQ ID NO: 33 - protein, 214 aa, Artificial Sequence
  Light chain variable region
DIQMTQSPSSLSASVGDRVTITCRASQDISNYLNWYQQKPGKAPKLLLYYTSRLHSGVPSRFSGSGSGTDYTLTISSLQPEDIATYFCQQGAGFPYTFGGGTKVEIKRTVAAPSVFIFPPSDEQLKSGTASVVCLLNNFYPREAKVQWKVDNALQSGNSQESVTEQDSKDSTYSLSSTLTLSKADYEKHKVYACEVTHQGLSSPVTKSFNRGEC

SEQ ID NO: 34 - protein, 214 aa, Artificial Sequence
  Light chain variable region
DIQMTQSPSSLSASVGDRVTITCRASQDISNYLNWYQQKPGKAPKLLLYYTSRLHSGVPSRFSGSGSGTDYTLTISSLQPEDIATYFCQQGDTFPYTFGGGTKVEIKRTVAAPSVFIFPPSDEQLKSGTASVVCLLNNFYPREAKVQWKVDNALQSGNSQESVTEQDSKDSTYSLSSTLTLSKADYEKHKVYACEVTHQGLSSPVTKSFNRGEC

SEQ ID NO: 35 - protein, 112 aa, Artificial Sequence
  Light chain variable region of hu5F9
DIVMTQSPLSLPVTPGEPASISCRSSQSIVYSNGNTYLGWYLQKPGQSPQLLIYKVSNRFSGVPDRFSGSGSGTDFTLKISRVEAEDVGVYYCFQGSHVPYTFGQGTKLEIK

SEQ ID NO: 36 - protein, 117 aa, Artificial Sequence
  Heavy chain variable region of hu5F9
QVQLVQSGAEVKKPGASVKVSCKASGYTFTNYNMHWVRQAPGQRLEWMGTIYPGNDDTSYNQKFKDRVTITADTSASTAYMELSSLRSEDTAVYYCARGGYRAMDYWGQGTLVTVSS

SEQ ID NO: 37 - protein, 113 aa, Artificial Sequence
  Light chain variable region of 1F8
DIVMTQSPDSLAVSLGERATINCKSSQSVLYSSNNRNYLAWYQQKPGQPPKLLINQASTRASGVPDRFSGSGSGTEFTLIISSLHAEDVAIYYCQQYYTPPLAFGGGTKLEIK

SEQ ID NO: 38 - protein, 118 aa, Artificial Sequence
  Heavy chain variable region of 1F8
KVQLVESGGGLVKPGGSLRLSCAASGFTFSNAWMNWVRQAPGKGLEWVGRIKRKTDGETTDYAAPVKGRFSISRDDSKNTLYLQMNSLKTEDTAVYYCAGSNRAFDIWGQGTMVTVSA

SEQ ID NO: 39 - protein, 327 aa, Artificial Sequence
  hz140-H-knobs, A chain Fc
ASTKGPSVFPLAPCSRSTSESTAALGCLVKDYFPEPVTVSWNSGALTSGVHTFPAVLQSSGLYSLSSVVTVPSSSLGTQTYTCNVDHKPSNTKVDKRVESKYGPPCPPCPAPEFLGGPSVFLFPPKPKDTLMISRTPEVTCVVVDVSQEDPEVQFNWYVDGVEVHNAKTKPREEQYNSTYRVVSVLTVLHQDWLNGKEYKCKVSNKGLPSSIEKTISKAKGQPREPQVYTLPPSQKEMTKNQVSLTCLVKGFYPSDIAVEWESNGQPENNYKTTPPVLDSDGSFFLYSKLTVDKSRWQEGNVFSCSVMHEALHNRYTQKSLSLSLGK

SEQ ID NO: 40 - protein, 451 aa, Artificial Sequence
  hz140-H-A
EVQLVQSGAEVKKPGASVKVSCKASGYKFTNYVMSWVRQAPGQRLEWMGYINPYNDAIKYNEKFTGRVTITRDTSASTAYMELSSLRSEDTAVYYCAREGDFYANYGRLGFAYWGQGTLVTVSSASTKGPSVFPLAPCSRSTSESTAALGCLVKDYFPEPVTVSWNSGALTSGVHTFPAVLQSSGLYSLSSVVTVPSSSLGTQTYTCNVDHKPSNTKVDKRVESKYGPPCPPCPAPEFLGGPSVFLFPPKPKDTLMISRTPEVTCVVVDVSQEDPEVQFNWYVDGVEVHNAKTKPREEQYNSTYRVVSVLTVLHQDWLNGKEYKCKVSNKGLPSSIEKTISKAKGQPREPQVYTLPPSQKEMTKNQVSLTCLVKGFYPSDIAVEWESNGQPENNYKTTPPVLDSDGSFFLYSKLTVDKSRWQEGNVFSCSVMHEALHNRYTQKSLSLSLGK

SEQ ID NO: 41 - protein, 327 aa, Artificial Sequence
  hz182-H-holes, B chain Fc
ASTKGPSVFPLAPCSRSTSESTAALGCLVKDYFPEPVTVSWNSGALTSGVHTFPAVLQSSGLYSLSSVVTVPSSSLGTQTYTCNVDHKPSNTKVDKRVESKYGPPCPPCPAPEFLGGPSVFLFPPKPKDTLMISRTPEVTCVVVDVSQEDPEVQFNWYVDGVEVHNAKTKPREEQYNSTYRVVSVLTVLHQDWLNGKEYKCKVSNKGLPSSIEKTISKAKGQPREPQVYTLPPSQEEMTKNQVSLTCLVKGFYPSDIAVEWESNGQPENNYKTTPPVLDSDGSFFLYSKLTVDKSRWQEGNVFSCSVMHEALHNHYTQESLSLSLGK

SEQ ID NO: 42 - protein, 446 aa, Artificial Sequence
  hz182-H-B
EVQLVQSGAEVKKPGATVKISCKVSGFNIKDIYMHWVQQAPGKGLEWMGRIDPANANTKYDPKFQDRVTITADTSTNTAYMELSSLRSEDTAVYYCASGQLGPLGFDYWGQGTTVTVSSASTKGPSVFPLAPCSRSTSESTAALGCLVKDYFPEPVTVSWNSGALTSGVHTFPAVLQSSGLYSLSSVVTVPSSSLGTQTYTCNVDHKPSNTKVDKRVESKYGPPCPPCPAPEFLGGPSVFLFPPKPKDTLMISRTPEVTCVVVDVSQEDPEVQFNWYVDGVEVHNAKTKPREEQYNSTYRVVSVLTVLHQDWLNGKEYKCKVSNKGLPSSIEKTISKAKGQPREPQVYTLPPSQEEMTKNQVSLTCLVKGFYPSDIAVEWESNGQPENNYKTTPPVLDSDGSFFLYSKLTVDKSRWQEGNVFSCSVMHEALHNHYTQESLSLSLGK

SEQ ID NO: 43 - protein, 108 aa, Artificial Sequence
  Light chain variable region of murine antibody 140
DIQMTQTTSSLSASLGDRVTISCRASQDITNYLNWYQQKPDGTVKLLIYYTSRLHSGVPSRFSGSGSGTDYSLTITNLEQEDIATYFCQQGDTFPRTFGGGTKLEIKR

SEQ ID NO: 44 - protein, 124 aa, Artificial Sequence
  Heavy chain variable region of murine antibody 140
EVQLQQSGPELIKPGPSVKMSCKASGYKFTNYVMHWVKQKPGQGLEWIGYINPYNDGIKYNEKFTGKATLTSDKSSNTAYMELISLTSEDSAVYYCAREGDFYANYGRLGFAYWGQGTLVTVSA

SEQ ID NO: 45 - protein, 23 aa, Artificial Sequence
  FR1
DIQMTQSPSSLSASVGDRVTITC

SEQ ID NO: 46 - protein, 11 aa, Artificial Sequence
  LCDR1
RASQDITNYLN

SEQ ID NO: 47 - protein, 11 aa, Artificial Sequence
  LCDR1
RASQDISNYLN

SEQ ID NO: 48 - protein, 15 aa, Artificial Sequence
  FR2
WYQQKPGKAPKLLIY

SEQ ID NO: 49 - protein, 15 aa, Artificial Sequence
  FR2
WYQQKPGKAPKLLLY

SEQ ID NO: 50 - protein, 7 aa, Artificial Sequence
  CDR2
YTSRLHS

SEQ ID NO: 51 - protein, 7 aa, Artificial Sequence
  CDR2
YTSRLSS

SEQ ID NO: 52 - protein, 7 aa, Artificial Sequence
  CDR2
YTSRLQS

SEQ ID NO: 53 - protein, 32 aa, Artificial Sequence
  FR3
GVPSRFSGSGSGTDYTFTISSLQPEDIATYFC

SEQ ID NO: 54 - protein, 32 aa, Artificial Sequence
  FR3
GVPSRFSGSGSGTDYTLTISSLQPEDIATYFC

SEQ ID NO: 55 - protein, 32 aa, Artificial Sequence
  FR3
GVPSRFSGSGSGTDYTFTISSLQPEDFATYFC

SEQ ID NO: 56 - protein, 9 aa, Artificial Sequence
  LCDR3
QQGDTFPRT

SEQ ID NO: 57 - protein, 9 aa, Artificial Sequence
  LCDR3
QQGATFPRT

SEQ ID NO: 58 - protein, 9 aa, Artificial Sequence
  LCDR3
QQGDGFPRT

SEQ ID NO: 59 - protein, 9 aa, Artificial Sequence
  LCDR3
QQGDTRPRT

SEQ ID NO: 60 - protein, 9 aa, Artificial Sequence
  LCDR3
QQGDTRPYT

SEQ ID NO: 61 - protein, 9 aa, Artificial Sequence
  LCDR3
QQGAGRPRT

SEQ ID NO: 62 - protein, 9 aa, Artificial Sequence
  LCDR3
QQGAGRPYT

SEQ ID NO: 63 - protein, 9 aa, Artificial Sequence
  LCDR3
QQGDTFPYT

SEQ ID NO: 64 - protein, 9 aa, Artificial Sequence
  LCDR3
QQGDTYPYT

SEQ ID NO: 65 - protein, 9 aa, Artificial Sequence
  LCDR3
QQGDTKPYT

SEQ ID NO: 66 - protein, 9 aa, Artificial Sequence
  LCDR3
QQGDTSPYT

SEQ ID NO: 67 - protein, 9 aa, Artificial Sequence
  LCDR3
QQGDTEPYT

SEQ ID NO: 68 - protein, 9 aa, Artificial Sequence
  LCDR3
QQGDTNPYT

SEQ ID NO: 69 - protein, 32 aa, Artificial Sequence
  FR3
GVPSRFSGSGSGTDYTLTISSLQPEDFATYFC

SEQ ID NO: 70 - protein, 9 aa, Artificial Sequence
  CDR3
QQGDGRPYT

SEQ ID NO: 71 - protein, 9 aa, Artificial Sequence
  CDR3
QQGATRPYT

SEQ ID NO: 72 - protein, 9 aa, Artificial Sequence
  CDR3
QQGAGFPYT

SEQ ID NO: 73 - protein, 30 aa, Artificial Sequence
  FR1
QVQLVQSGAEVKKPGASVKVSCKASGYKFT

SEQ ID NO: 74 - protein, 30 aa, Artificial Sequence
  FR1
QVQLVQSGAEVKKPGASVKVSCKASGYTFT

SEQ ID NO: 75 - protein, 30 aa, Artificial Sequence
  FR1
EVQLVQSGAEVKKPGASVKVSCKASGYKFT

SEQ ID NO: 76 - protein, 5 aa, Artificial Sequence
  CDR1
NYVMH

SEQ ID NO: 77 - protein, 5 aa, Artificial Sequence
  CDR1
SYVMH

SEQ ID NO: 78 - protein, 5 aa, Artificial Sequence
  CDR1
NYVMS

SEQ ID NO: 79 - protein, 17 aa, Artificial Sequence
  CDR2
YINPYNDGIKYNEKFTG

SEQ ID NO: 80 - protein, 17 aa, Artificial Sequence
  CDR2
WINPYNDGIKYNEKFTG

SEQ ID NO: 81 - protein, 17 aa, Artificial Sequence
  CDR2
YINPGNDGIKYNEKFTG

SEQ ID NO: 82 - protein, 17 aa, Artificial Sequence
  CDR2
YINPYNDGIKYNEKFQG

SEQ ID NO: 83 - protein, 17 aa, Artificial Sequence
  CDR2
YINPYNDAIKYNEKFTG

SEQ ID NO: 84 - protein, 17 aa, Artificial Sequence
  CDR2
YINPYNEGIKYNEKFTG

SEQ ID NO: 85 - protein, 15 aa, Artificial Sequence
  CDR3
EGDFYANYGRLGFAY

SEQ ID NO: 86 - protein, 15 aa, Artificial Sequence
  CDR3
EGDFYANYGRLGFDY

SEQ ID NO: 87 - protein, 5 aa, Artificial Sequence
  CDR1
NYAMH